European Patent Application EP 4 606 896 A1, published August 27, 2025. Title: 抗体、核酸、細胞、及び医薬. Applicant: 株式会社エヌビィー健康研究所. The sequence listing filed with the application follows.

SEQUENCE LISTING (130 sequences)

SEQ ID NO: 1 - protein, 10 aa, Mus musculus
GYTFTSYGIS

SEQ ID NO: 2 - protein, 17 aa, Mus musculus
EIYPRSGNTYYNEKFKG

SEQ ID NO: 3 - protein, 15 aa, Mus musculus
ARESISRRLGWNFDV

SEQ ID NO: 4 - protein, 11 aa, Mus musculus
RASENIYSFLA

SEQ ID NO: 5 - protein, 7 aa, Mus musculus
NAKTLTE

SEQ ID NO: 6 - protein, 9 aa, Mus musculus
QHHYGPPLT

SEQ ID NO: 7 - protein, 122 aa, Mus musculus
QVQLQQSGAELARPGASVKLSCKASGYTFTSYGISWVKQRTGQGLEWIGEIYPRSGNTYYNEKFKGKATLTADKSSSTAYMELRSLTSEDSAVYFCARESISRRLGWNFDVWGTGTTVTVSS

SEQ ID NO: 8 - DNA, 366 bp, Mus musculus
  source 1..366: mol_type = other DNA
  CDS 1..366: protein_id = 7; translation = QVQLQQSGAELARPGASVKLSCKASGYTFTSYGISWVKQRTGQGLEWIGEIYPRSGNTYYNEKFKGKATLTADKSSSTAYMELRSLTSEDSAVYFCARESISRRLGWNFDVWGTGTTVTVSS
caggttcagctgcagcagtctggagctgagctggcgaggcctggggcttcagtgaagctgtcctgcaaggcttctggctacaccttcacaagctatggtataagctgggtgaagcagagaactggacagggccttgagtggattggagagatttatcctagaagtggtaatacttactacaatgagaagttcaagggcaaggccacactgactgcagacaaatcctccagcacagcgtacatggagctccgcagcctgacatctgaggactctgcggtctatttctgtgcaagagagtctatatcacgacggctaggctggaacttcgatgtctggggcacagggaccacggtcaccgtctcctca

SEQ ID NO: 9 - protein, 107 aa, Mus musculus
DIHMTQSPASLSASVGETVTITCRASENIYSFLAWYQQKQGKSPHLVVYNAKTLTEGVPSRFSGSGSGTHFSLKINSLQPEDFGIYYCQHHYGPPLTFGAGTKLELK

SEQ ID NO: 10 - DNA, 321 bp, Mus musculus
  source 1..321: mol_type = other DNA
  CDS 1..321: protein_id = 9; translation = DIHMTQSPASLSASVGETVTITCRASENIYSFLAWYQQKQGKSPHLVVYNAKTLTEGVPSRFSGSGSGTHFSLKINSLQPEDFGIYYCQHHYGPPLTFGAGTKLELK
gacatccacatgactcagtctccagcctccctatctgcatctgtgggagaaactgtcaccatcacatgtcgagcaagtgagaatatttacagttttttagcatggtatcagcagaaacagggaaaatctcctcacctcgtggtctacaatgcaaagaccttaacagaaggtgtgccatcaaggttcagtggcagtggatcaggcacacacttttctctgaagatcaacagccttcagcctgaagattttgggatttattactgtcaacatcattatggtcctcctctcacgttcggtgctgggaccaagctggagctgaaa

SEQ ID NO: 11 - protein, 10 aa, Mus musculus
GYSFTAYGIS

SEQ ID NO: 12 - protein, 17 aa, Mus musculus
EIYPRSGNTYYSEKFKG

SEQ ID NO: 13 - protein, 15 aa, Mus musculus
ARESLLKRLGWYFDV

SEQ ID NO: 14 - protein, 11 aa, Mus musculus
RASQNIYSFLA

SEQ ID NO: 15 - protein, 7 aa, Mus musculus
NAKTLAE

SEQ ID NO: 16 - protein, 9 aa, Mus musculus
QHHYGPPLT

SEQ ID NO: 17 - protein, 122 aa, Mus musculus
QVHLQQSGAELARPGASVKLSCKASGYSFTAYGISWVQQRTGQGLEWIGEIYPRSGNTYYSEKFKGKATLTADKSSSTAYMELRSLTSEDSAVYFCARESLLKRLGWYFDVWGTGTTVTVSS

SEQ ID NO: 18 - DNA, 366 bp, Mus musculus
  source 1..366: mol_type = other DNA
  CDS 1..366: protein_id = 17; translation = QVHLQQSGAELARPGASVKLSCKASGYSFTAYGISWVQQRTGQGLEWIGEIYPRSGNTYYSEKFKGKATLTADKSSSTAYMELRSLTSEDSAVYFCARESLLKRLGWYFDVWGTGTTVTVSS
caggttcatctgcagcagtctggagctgagctggcgaggcctggggcttcagtgaagctgtcctgcaaggcttctggctacagcttcacagcctatggtataagctgggtgcagcagagaactggacagggccttgagtggattggagagatttatccaagaagtggtaatacttactacagtgagaagttcaagggcaaggccacactgactgcagacaaatcctccagtacagcgtacatggagctccgcagcctgacatctgaggactctgcggtctatttctgtgcaagagagtctctattaaaacggctaggctggtacttcgatgtctggggcacagggaccacggtcaccgtctcctca

SEQ ID NO: 19 - protein, 107 aa, Mus musculus
DIQMTQSPASLSASVGETVTITCRASQNIYSFLAWYQQKQGNSPQLLVYNAKTLAEGVPSRFSGSGSGTQFSLKINSLQPEDFGSYYCQHHYGPPLTFGVGTKLELK

SEQ ID NO: 20 - DNA, 321 bp, Mus musculus
  source 1..321: mol_type = other DNA
  CDS 1..321: protein_id = 19; translation = DIQMTQSPASLSASVGETVTITCRASQNIYSFLAWYQQKQGNSPQLLVYNAKTLAEGVPSRFSGSGSGTQFSLKINSLQPEDFGSYYCQHHYGPPLTFGVGTKLELK
gacatccagatgactcagtctccagcctccctatctgcatctgtgggagaaactgtcaccatcacatgtcgagcaagtcagaatatttacagttttttagcatggtatcagcagaaacagggaaattctcctcagctcctggtctataatgcaaaaaccttagcagaaggtgtgccatcaaggttcagtggcagtggatcaggcacacagttttctctgaagatcaacagcctgcagcctgaagattttgggagttattactgtcaacatcattatggtcctcctctcacgttcggtgttgggaccaagctggagctgaaa

SEQ ID NO: 21 - protein, 10 aa, Mus musculus
GYTFTSYGIS

SEQ ID NO: 22 - protein, 17 aa, Mus musculus
EIYPRSGVTYYNEKFKG

SEQ ID NO: 23 - protein, 15 aa, Mus musculus
ARESISLRLGWYFDV

SEQ ID NO: 24 - protein, 11 aa, Mus musculus
RASENIYRFLA

SEQ ID NO: 25 - protein, 7 aa, Mus musculus
NAKTLAE

SEQ ID NO: 26 - protein, 9 aa, Mus musculus
QHHYGPPLT

SEQ ID NO: 27 - protein, 122 aa, Mus musculus
QVQLQQSGAELARPGASMKLSCRASGYTFTSYGISWVKQRTGQGLEWIGEIYPRSGVTYYNEKFKGRATLTADKSSSTAFMELRSLTSEDSAVYFCARESISLRLGWYFDVWGTGTTVTVSS

SEQ ID NO: 28 - DNA, 366 bp, Mus musculus
  source 1..366: mol_type = other DNA
  CDS 1..366: protein_id = 27; translation = QVQLQQSGAELARPGASMKLSCRASGYTFTSYGISWVKQRTGQGLEWIGEIYPRSGVTYYNEKFKGRATLTADKSSSTAFMELRSLTSEDSAVYFCARESISLRLGWYFDVWGTGTTVTVSS
caggttcagctgcagcagtctggagctgagctggcgaggcctggggcttcaatgaagctgtcctgcagggcttctggctacaccttcacaagctatggtataagctgggtgaagcagagaactggacagggccttgagtggattggagagatttatcccagaagtggtgttacttactacaatgagaagttcaagggtagggccacactgactgcagacaaatcctccagcacagcgttcatggagctccgcagcctgacatctgaggactctgcggtctatttctgtgcaagagagtctatatcactacgactaggctggtacttcgatgtctggggcacagggaccacggtcaccgtctcctca

SEQ ID NO: 29 - protein, 107 aa, Mus musculus
DIQMTQSPASLSASVGDTVTITCRASENIYRFLAWYQQKQRKSPHLLVYNAKTLAEGVPSRFSGSGSGTQFSLKINSLQPEDFGSYYCQHHYGPPLTFGAGTKLELT

SEQ ID NO: 30 - DNA, 321 bp, Mus musculus
  source 1..321: mol_type = other DNA
  CDS 1..321: protein_id = 29; translation = DIQMTQSPASLSASVGDTVTITCRASENIYRFLAWYQQKQRKSPHLLVYNAKTLAEGVPSRFSGSGSGTQFSLKINSLQPEDFGSYYCQHHYGPPLTFGAGTKLELT
gacatccagatgactcagtctccagcctccctatctgcatctgtgggagatactgtcaccatcacatgtcgagcaagtgagaatatttacaggtttttagcatggtatcagcagaaacagagaaaatctccgcacctcctggtctataatgcaaaaaccttagcagaaggtgtgccatcaaggttcagtggcagtggatcaggcacacagttttctctgaagatcaacagtctgcagcctgaagattttgggagttattattgtcaacatcattatggtcctccactcacgttcggtgctgggaccaagctggagctgaca

SEQ ID NO: 31 - protein, 10 aa, Mus musculus
GYTFTSYGIS

SEQ ID NO: 32 - protein, 17 aa, Mus musculus
EIYPRSGNTYYNEKFKG

SEQ ID NO: 33 - protein, 15 aa, Mus musculus
ARESILLRLGWYFDV

SEQ ID NO: 34 - protein, 11 aa, Mus musculus
RASENIYRFLA

SEQ ID NO: 35 - protein, 7 aa, Mus musculus
NAKTLAE

SEQ ID NO: 36 - protein, 9 aa, Mus musculus
QHHYGPPLT

SEQ ID NO: 37 - protein, 122 aa, Mus musculus
QVQLQQSGAELARPGASVKLSCKASGYTFTSYGISWVKQRTGQGLEWIGEIYPRSGNTYYNEKFKGRATLTADKSSSTAYMELRSLTSEDSAVYFCARESILLRLGWYFDVWGTGTTVTVSS

SEQ ID NO: 38 - DNA, 366 bp, Mus musculus
  source 1..366: mol_type = other DNA
  CDS 1..366: protein_id = 37; translation = QVQLQQSGAELARPGASVKLSCKASGYTFTSYGISWVKQRTGQGLEWIGEIYPRSGNTYYNEKFKGRATLTADKSSSTAYMELRSLTSEDSAVYFCARESILLRLGWYFDVWGTGTTVTVSS
caggttcagctgcagcagtctggagctgagctggcgaggcctggggcttcagtgaagctgtcctgcaaggcttctggctacaccttcacaagctatggtataagctgggtgaagcagagaactggacagggccttgagtggattggagagatttatcctagaagtggtaatacttactacaatgagaagttcaagggcagggccacactgactgcagacaaatcctccagcacagcgtacatggagctccgcagcctgacatctgaggactctgcggtctatttctgtgcaagagagtctatattactacggctaggctggtacttcgatgtctggggcacagggaccacggtcaccgtctcctca

SEQ ID NO: 39 - protein, 107 aa, Mus musculus
DIQMTQSPASLSASVGGTVTITCRASENIYRFLAWYQQKQGKSPQLLVYNAKTLAEGVPSRFSGSGSGTQFSLKINSLQPEDFGIYYCQHHYGPPLTFGAGTKLELK

SEQ ID NO: 40 - DNA, 321 bp, Mus musculus
  source 1..321: mol_type = other DNA
  CDS 1..321: protein_id = 39; translation = DIQMTQSPASLSASVGGTVTITCRASENIYRFLAWYQQKQGKSPQLLVYNAKTLAEGVPSRFSGSGSGTQFSLKINSLQPEDFGIYYCQHHYGPPLTFGAGTKLELK
gacatccagatgactcagtctccagcctccctatctgcatctgtgggaggaactgtcaccatcacatgtcgagcaagtgagaatatttacaggtttttagcatggtatcagcagaaacagggaaaatctcctcagctcctggtctataatgcaaaaaccttagcagaaggtgtgccatcaaggttcagtggcagtggatcaggcacacagttttctctgaagatcaacagccttcagcctgaagattttgggatttattactgtcaacatcattatggtcctcctctcacgttcggtgctgggaccaagctggagctgaaa

SEQ ID NO: 41 - protein, 10 aa, Mus musculus
GYTFTSYGIS

SEQ ID NO: 42 - protein, 17 aa, Mus musculus
EIYPRSGNTYYNEKVKG

SEQ ID NO: 43 - protein, 15 aa, Mus musculus
ARESIFLRLGWYFDV

SEQ ID NO: 44 - protein, 11 aa, Mus musculus
RASDNIYRFLA

SEQ ID NO: 45 - protein, 7 aa, Mus musculus
NAKTLAE

SEQ ID NO: 46 - protein, 9 aa, Mus musculus
QHHYGPPLT

SEQ ID NO: 47 - protein, 122 aa, Mus musculus
QVQLQQSGAELARPGASVKLSCKASGYTFTSYGISWVKQRTGQGLEWIGEIYPRSGNTYYNEKVKGKATLTADKSSSTAYMELRSLTSEDSAVYFCARESIFLRLGWYFDVWGTGTTVTVSS

SEQ ID NO: 48 - DNA, 366 bp, Mus musculus
  source 1..366: mol_type = other DNA
  CDS 1..366: protein_id = 47; translation = QVQLQQSGAELARPGASVKLSCKASGYTFTSYGISWVKQRTGQGLEWIGEIYPRSGNTYYNEKVKGKATLTADKSSSTAYMELRSLTSEDSAVYFCARESIFLRLGWYFDVWGTGTTVTVSS
caggttcagctgcagcagtctggagctgagctggcgaggcctggggcttcagtgaagctgtcctgcaaggcttctggctacaccttcacaagctatggtataagttgggtgaagcagagaactggacagggccttgagtggattggagagatttatcctagaagtggtaatacttactacaatgagaaggtcaagggcaaggccacactgactgcagacaaatcctccagcacagcgtacatggagctccgcagcctgacatctgaggactctgcggtctatttctgtgcaagagagtctatattcctacgtctaggctggtacttcgatgtctggggcacagggaccacggtcaccgtctcctca

SEQ ID NO: 49 - protein, 107 aa, Mus musculus
DIQMTQSPASLSASVGETVTITCRASDNIYRFLAWYQQKQGKSPQLLVYNAKTLAEGVPSRFSGSGTGTQFSLKINSLQPEDFGIYYCQHHYGPPLTFGAGTKLELK

SEQ ID NO: 50 - DNA, 321 bp, Mus musculus
  source 1..321: mol_type = other DNA
  CDS 1..321: protein_id = 49; translation = DIQMTQSPASLSASVGETVTITCRASDNIYRFLAWYQQKQGKSPQLLVYNAKTLAEGVPSRFSGSGTGTQFSLKINSLQPEDFGIYYCQHHYGPPLTFGAGTKLELK
gacatccagatgactcagtctccagcctccctatctgcatctgtgggagaaactgtcaccatcacatgtcgagcaagtgacaatatttacaggtttttagcatggtatcagcagaaacagggaaaatctcctcagctcctggtctataatgcaaaaaccttagcagaaggtgtgccatcaaggttcagtggcagtggaacaggcacacagttttctctgaagatcaacagtcttcagcctgaagattttgggatttattactgtcaacatcattatggtcctcctctcacgttcggtgctgggaccaagctggagctgaaa

SEQ ID NO: 51 - protein, 10 aa, Mus musculus
GYTFTSFGVN

SEQ ID NO: 52 - protein, 17 aa, Mus musculus
QIYPRTGTTYHNERFKG

SEQ ID NO: 53 - protein, 11 aa, Mus musculus
AREGDRYSLAY

SEQ ID NO: 54 - protein, 11 aa, Mus musculus
RASENIYRFLA

SEQ ID NO: 55 - protein, 7 aa, Mus musculus
NAKTLVE

SEQ ID NO: 56 - protein, 9 aa, Mus musculus
QHHYGIPLT

SEQ ID NO: 57 - protein, 118 aa, Mus musculus
QVQVQQSGAELARPGASVRLSCKASGYTFTSFGVNWVKQRTGQGLEWIGQIYPRTGTTYHNERFKGKATLTTDKSSSTAYMELRSLTSEDSAVYFCAREGDRYSLAYWGQGTLVTVSA

SEQ ID NO: 58 - DNA, 354 bp, Mus musculus
  source 1..354: mol_type = other DNA
  CDS 1..354: protein_id = 57; translation = QVQVQQSGAELARPGASVRLSCKASGYTFTSFGVNWVKQRTGQGLEWIGQIYPRTGTTYHNERFKGKATLTTDKSSSTAYMELRSLTSEDSAVYFCAREGDRYSLAYWGQGTLVTVSA
caggttcaggtacagcagtccggagctgagctggcgaggcctggggcatcagtgaggctgtcctgcaaggcttctggctacaccttcacaagctttggtgtaaactgggtgaagcagagaactggacagggccttgagtggattggacagatttatcctagaactggtactacttaccacaatgagaggttcaagggcaaggccacactgactacagacaaatcctccagcacagcgtacatggagctccgcagcctgacatctgaggactctgcggtctatttctgtgcacgagagggagataggtactcacttgcttactggggccaagggactctggtcactgtctctgca

SEQ ID NO: 59 - protein, 107 aa, Mus musculus
DIQMTQSPASLSASVGETVTITCRASENIYRFLAWYQQKQGKSPQLLVYNAKTLVEGVPSRFSGSGSGTQFSLKINNLQPEDFGSYYCQHHYGIPLTFGAGTKLELK

SEQ ID NO: 60 - DNA, 321 bp, Mus musculus
  source 1..321: mol_type = other DNA
  CDS 1..321: protein_id = 59; translation = DIQMTQSPASLSASVGETVTITCRASENIYRFLAWYQQKQGKSPQLLVYNAKTLVEGVPSRFSGSGSGTQFSLKINNLQPEDFGSYYCQHHYGIPLTFGAGTKLELK
gacatccagatgactcagtctccagcctccctatctgcatctgtgggagaaactgtcaccatcacatgtcgagcaagtgagaatatttacaggtttttagcatggtatcagcagaaacagggaaaatctcctcagctcctggtctataatgcaaaaaccttagtagaaggtgtgccatcaaggttcagtggcagtggatcaggcacacagttttctctgaagatcaacaacctacagcctgaagattttgggagttattactgtcaacatcattatggtattccgctcacgttcggtgctgggaccaagctggagctgaaa

SEQ ID NO: 61 - protein, 10 aa, Mus musculus
GYTFASFGIS

SEQ ID NO: 62 - protein, 17 aa, Mus musculus
EIYPRSGTTYFNEKFRG

SEQ ID NO: 63 - protein, 12 aa, Mus musculus
AREGVRRYAMDY

SEQ ID NO: 64 - protein, 11 aa, Mus musculus
RASGNIYSFLA

SEQ ID NO: 65 - protein, 7 aa, Mus musculus
NAKTLAE

SEQ ID NO: 66 - protein, 9 aa, Mus musculus
QHHYGIPLT

SEQ ID NO: 67 - protein, 119 aa, Mus musculus
QLHLQQSGAELARPGASVRLSCKASGYTFASFGISWVKQRTGQGLEYIGEIYPRSGTTYFNEKFRGKATLSADKSSSTAYMELRSLTSEDSAVYFCAREGVRRYAMDYWGQGTSVTVSS

SEQ ID NO: 68 - DNA, 357 bp, Mus musculus
  source 1..357: mol_type = other DNA
  CDS 1..357: protein_id = 67; translation = QLHLQQSGAELARPGASVRLSCKASGYTFASFGISWVKQRTGQGLEYIGEIYPRSGTTYFNEKFRGKATLSADKSSSTAYMELRSLTSEDSAVYFCAREGVRRYAMDYWGQGTSVTVSS
cagcttcacctgcagcagtctggagctgagctggcgaggcctggggcttcagtgaggctgtcctgcaaggcttctggctacaccttcgcaagttttggtataagctgggtgaagcagagaactggacagggccttgaatacattggagagatttatcctagaagtggtactacttacttcaatgagaagttcaggggcaaggccacactgagtgcagacaaatcatccagcacagcgtacatggagctccgcagcctgacatctgaggactctgcggtctatttctgtgcaagagagggagtacgacggtatgctatggactactggggtcaaggaacctcagtcaccgtctcctca

SEQ ID NO: 69 - protein, 107 aa, Mus musculus
DIQVTQSPASLSASVGETVTITCRASGNIYSFLAWYQQKQGKSPQLLVYNAKTLAEGVPSRFSGSGSGTQFSLKISSLQPEDFGSYYCQHHYGIPLTFGAGTKLDLK

SEQ ID NO: 70 - DNA, 321 bp, Mus musculus
  source 1..321: mol_type = other DNA
  CDS 1..321: protein_id = 69; translation = DIQVTQSPASLSASVGETVTITCRASGNIYSFLAWYQQKQGKSPQLLVYNAKTLAEGVPSRFSGSGSGTQFSLKISSLQPEDFGSYYCQHHYGIPLTFGAGTKLDLK
gacatccaggtgactcagtctccagcctccctatctgcgtctgtgggagaaactgtcaccatcacatgtcgcgcaagtgggaatatttacagttttttagcatggtatcagcagaaacagggaaaatctcctcaactcctggtctataatgcaaaaactttagcagaaggtgtgccatcaaggttcagtggcagtggatcaggcacacagttttctctgaagatcagcagcctgcagcctgaagattttgggagttattactgtcaacatcattatggtattcctctcacgttcggtgctgggaccaagttggacctgaaa

SEQ ID NO: 71 - protein, 10 aa, Mus musculus
GYTFASFGIS

SEQ ID NO: 72 - protein, 17 aa, Mus musculus
EIYPRSGTTYFNEKFRG

SEQ ID NO: 73 - protein, 12 aa, Mus musculus
AREGVRRYAMDY

SEQ ID NO: 74 - protein, 11 aa, Mus musculus
RASGNIYSFLA

SEQ ID NO: 75 - protein, 7 aa, Mus musculus
NAKTLAE

SEQ ID NO: 76 - protein, 9 aa, Mus musculus
QHHYGIPLT

SEQ ID NO: 77 - protein, 119 aa, Mus musculus
QFQLQQSGAELARPGASVKLSCKASGYTFASFGISWVKQRTGQGLEYIGEIYPRSGTTYFNEKFRGKATLTADKSSSTAYMELRSLTSEDSAVYFCAREGVRRYAMDYWGQGTSVTVSS

SEQ ID NO: 78 - DNA, 357 bp, Mus musculus
  source 1..357: mol_type = other DNA
  CDS 1..357: protein_id = 77; translation = QFQLQQSGAELARPGASVKLSCKASGYTFASFGISWVKQRTGQGLEYIGEIYPRSGTTYFNEKFRGKATLTADKSSSTAYMELRSLTSEDSAVYFCAREGVRRYAMDYWGQGTSVTVSS
cagtttcagctgcagcagtctggagctgagctggcgaggcctggggcttcagtgaagctgtcctgcaaggcttctggctacaccttcgcaagctttggtataagctgggtgaaacagagaactggacagggccttgaatacattggagagatttatcctagaagtggtactacttacttcaatgagaaattcaggggcaaggccacactgactgcagacaaatcatccagcacagcgtacatggagctccgcagcctgacatctgaggactctgcggtctatttctgtgcaagagagggggtacgacggtatgctatggactactggggtcaaggaacctcagtcaccgtctcctca

SEQ ID NO: 79 - protein, 107 aa, Mus musculus
DIQVTQSPASLSASVGETVTITCRASGNIYSFLAWYQQKQGKSPQLLVYNAKTLAEGVPSRFSGSGSGTQFSLKISSLQPEDFGSYYCQHHYGIPLTFGGGTKLDLK

SEQ ID NO: 80 - DNA, 321 bp, Mus musculus
  source 1..321: mol_type = other DNA
  CDS 1..321: protein_id = 79; translation = DIQVTQSPASLSASVGETVTITCRASGNIYSFLAWYQQKQGKSPQLLVYNAKTLAEGVPSRFSGSGSGTQFSLKISSLQPEDFGSYYCQHHYGIPLTFGGGTKLDLK
gacatccaggtgactcagtctccagcctccctatctgcgtctgtgggagaaactgtcaccatcacatgtcgcgcaagtgggaatatttacagttttttagcatggtatcagcagaaacagggaaaatctcctcagctcctggtctataatgcaaaaaccttagcagaaggtgtgccatcaaggttcagtggcagtggatcaggcacacagttttctctgaagattagcagcctgcagcctgaagattttgggagttattactgtcaacatcattatggtattcctctcacgttcggtggtgggaccaagttggacctgaaa

SEQ ID NO: 81 - protein, 10 aa, Mus musculus
GYTFASFGIS

SEQ ID NO: 82 - protein, 17 aa, Mus musculus
EIYPRSGTTYFNEKFRG

SEQ ID NO: 83 - protein, 12 aa, Mus musculus
AREGVRRYAMDY

SEQ ID NO: 84 - protein, 11 aa, Mus musculus
RASGNIYSFLA

SEQ ID NO: 85 - protein, 7 aa, Mus musculus
NAKTLAE

SEQ ID NO: 86 - protein, 9 aa, Mus musculus
QHHYGIPLT

SEQ ID NO: 87 - protein, 119 aa, Mus musculus
QLQLQQSGAELARPGASVKLSCKASGYTFASFGISWVKQRAGQGLEYIGEIYPRSGTTYFNEKFRGKATLTADKSSSTAYMELRRLTSEDSAVYFCAREGVRRYAMDYWGQGTSVTVSS

SEQ ID NO: 88 - DNA, 357 bp, Mus musculus
  source 1..357: mol_type = other DNA
  CDS 1..357: protein_id = 87; translation = QLQLQQSGAELARPGASVKLSCKASGYTFASFGISWVKQRAGQGLEYIGEIYPRSGTTYFNEKFRGKATLTADKSSSTAYMELRRLTSEDSAVYFCAREGVRRYAMDYWGQGTSVTVSS
cagcttcagctgcagcagtctggagctgagctggcgaggcctggggcttcagtgaagctgtcctgcaaggcttctggctacaccttcgcaagttttggtataagttgggtgaagcagagagctggacagggccttgagtacattggagagatttatcctagaagtggtactacttacttcaatgagaagttcaggggcaaggccacactgactgcagacaaatcatccagcacagcgtacatggagctccgcagactgacatctgaggactctgcggtctatttctgtgcaagagagggggtacgacggtatgctatggactactggggtcaaggaacctcagtcaccgtctcctca

SEQ ID NO: 89 - protein, 107 aa, Mus musculus
DIQVTQSPASLSASVGETVTITCRASGNIYSFLAWYQQKQGKSPQLLVYNAKTLAEGVPSRFSGSGSGTQFSLKINSLQPEDFGSYYCQHHYGIPLTFGAGTKLDLK

SEQ ID NO: 90 - DNA, 321 bp, Mus musculus
  source 1..321: mol_type = other DNA
  CDS 1..321: protein_id = 89; translation = DIQVTQSPASLSASVGETVTITCRASGNIYSFLAWYQQKQGKSPQLLVYNAKTLAEGVPSRFSGSGSGTQFSLKINSLQPEDFGSYYCQHHYGIPLTFGAGTKLDLK
gacatccaggtgactcagtctccagcctccctatctgcgtctgtgggagaaactgtcaccatcacatgtcgcgcaagtgggaatatttacagttttttagcatggtatcagcagaaacagggaaaatctcctcagctcctggtctataatgcaaaaaccttagcagaaggtgtgccatcaaggttcagtggcagtggatcaggcacacagttttctctgaagatcaacagcctgcagcctgaagattttgggagttattactgtcaacatcattatggtattcctctcacgttcggtgctgggaccaagttggacctgaaa

SEQ ID NO: 91 - protein, 10 aa, Mus musculus
GYTFTSFGVN

SEQ ID NO: 92 - protein, 17 aa, Mus musculus
QIYPRTGTTYHNERFKG

SEQ ID NO: 93 - protein, 11 aa, Mus musculus
AREGDRYSLAY

SEQ ID NO: 94 - protein, 11 aa, Mus musculus
RASENIYRFLA

SEQ ID NO: 95 - protein, 7 aa, Mus musculus
NAKTLVE

SEQ ID NO: 96 - protein, 9 aa, Mus musculus
QHHYGIPLT

SEQ ID NO: 97 - protein, 118 aa, Mus musculus
QVQVQQSGAELARPGASVRLSCKASGYTFTSFGVNWVKQRTGQGLEWIGQIYPRTGTTYHNERFKGKATLTADKSSSTAYMELRSLTSEDSAVYFCAREGDRYSLAYWGQGTLVTVSA

SEQ ID NO: 98 - DNA, 354 bp, Mus musculus
  source 1..354: mol_type = other DNA
  CDS 1..354: protein_id = 97; translation = QVQVQQSGAELARPGASVRLSCKASGYTFTSFGVNWVKQRTGQGLEWIGQIYPRTGTTYHNERFKGKATLTADKSSSTAYMELRSLTSEDSAVYFCAREGDRYSLAYWGQGTLVTVSA
caggttcaggtacagcagtccggagctgagctggcgaggcctggggcatcagtgaggctgtcctgcaaggcttctggctacaccttcacaagttttggtgtaaactgggtgaagcagagaactggacagggccttgagtggattggacagatttatcctagaactggtactacttaccacaatgagaggttcaagggcaaggccacactgactgcagacaagtcctccagcacagcgtacatggagctccgcagcctgacatctgaggactctgcggtctatttctgtgcacgagagggagataggtactcacttgcttactggggccaagggactctggtcactgtctctgca

SEQ ID NO: 99 - protein, 107 aa, Mus musculus; identical to SEQ ID NO: 59

SEQ ID NO: 100 - DNA, 321 bp, Mus musculus; identical to SEQ ID NO: 60
  source 1..321: mol_type = other DNA
  CDS 1..321: protein_id = 99; translation = DIQMTQSPASLSASVGETVTITCRASENIYRFLAWYQQKQGKSPQLLVYNAKTLVEGVPSRFSGSGSGTQFSLKINNLQPEDFGSYYCQHHYGIPLTFGAGTKLELK

SEQ ID NO: 101 - protein, 10 aa, Mus musculus
GYTFTSFGVN

SEQ ID NO: 102 - protein, 17 aa, Mus musculus
QIYPRSGTTYHNERFKG

SEQ ID NO: 103 - protein, 11 aa, Mus musculus
AREGDRYSLAY

SEQ ID NO: 104 - protein, 11 aa, Mus musculus
RASENIYRFLA

SEQ ID NO: 105 - protein, 7 aa, Mus musculus
NAKTLAE

SEQ ID NO: 106 - protein, 9 aa, Mus musculus
QHHYGIPLT

SEQ ID NO: 107 - protein, 118 aa, Mus musculus
QVQVHQSGAELARPGASVRLSCKASGYTFTSFGVNWVKQRTGQGLEWIGQIYPRSGTTYHNERFKGKATLTADKSSSTAYMELRSLTSEDSAVYFCAREGDRYSLAYWGQGTLVTVSA

SEQ ID NO: 108 - DNA, 354 bp, Mus musculus
  source 1..354: mol_type = other DNA
  CDS 1..354: protein_id = 107; translation = QVQVHQSGAELARPGASVRLSCKASGYTFTSFGVNWVKQRTGQGLEWIGQIYPRSGTTYHNERFKGKATLTADKSSSTAYMELRSLTSEDSAVYFCAREGDRYSLAYWGQGTLVTVSA
caggttcaggtacaccagtccggagctgagctggcgaggcctggggcatcagtgaggctgtcctgcaaggcttctggctacaccttcacgagctttggtgtaaactgggtgaagcagagaactggacagggccttgagtggattggacagatttatcctagaagtggtactacttaccacaatgagaggttcaagggcaaggccacactgactgcagacaaatcctccagcacagcgtacatggagctccgcagcctgacatctgaggactctgcggtctatttctgtgcaagagagggagataggtactcacttgcttactggggccaagggactctggtcactgtctctgca

SEQ ID NO: 109 - protein, 107 aa, Mus musculus
DIQMTQSPASLSASVGETVTITCRASENIYRFLAWYQQKQGKSPQLLVSNAKTLAEGVPSRFSGSGSGTQFSLKINYLQPEDFGNYYCQHHYGIPLTFGAGTKLELK

SEQ ID NO: 110 - DNA, 321 bp, Mus musculus
  source 1..321: mol_type = other DNA
  CDS 1..321: protein_id = 109; translation = DIQMTQSPASLSASVGETVTITCRASENIYRFLAWYQQKQGKSPQLLVSNAKTLAEGVPSRFSGSGSGTQFSLKINYLQPEDFGNYYCQHHYGIPLTFGAGTKLELK
gacatccagatgactcagtctccagcctccctatctgcatctgtgggagaaactgtcaccatcacatgtcgagcaagtgagaatatttacaggtttttagcatggtatcagcagaaacagggaaaatctcctcagctcctggtctctaatgcaaaaaccttagcagaaggtgtgccatcaaggttcagtggcagtggatcaggcacacagttttctctgaagatcaactacctacagcctgaagattttgggaattattactgtcaacatcattatggtattccgctcacgttcggtgctgggaccaagctggagctgaaa

SEQ ID NO: 111 - protein, 364 aa, Homo sapiens
MAAISTSIPVISQPQFTAMNEPQCFYNESIAFFYNRSGKHLATEWNTVSKLVMGLGITVCIFIMLANLLVMVAIYVNRRFHFPIYYLMANLAAADFFAGLAYFYLMFNTGPNTRRLTVSTWLLRQGLIDTSLTASVANLLAIAIERHITVFRMQLHTRMSNRRVVVVIVVIWTMAIVMGAIPSVGWNCICDIENCSNMAPLYSDSYLVFWAIFNLVTFVVMVVLYAHIFGYVRQRTMRMSRHSSGPRRNRDTMMSLLKTVVIVLGAFIICWTPGLVLLLLDVCCPQCDVLAYEKFFLLLAEFNSAMNPIIYSYRDKEMSATFRQILCCQRSENPTGPTEGSDRSASSLNHTILAGVHSNDHSVV

SEQ ID NO: 112 - protein, 364 aa, Mus musculus
MAAASTSSPVISQPQFTAMNEQQCFYNESIAFFYNRSGKYLATEWNTVSKLVMGLGITVCVFIMLANLLVMVAIYVNRRFHFPIYYLMANLAAADFFAGLAYFYLMFNTGPNTRRLTVSTWLLRQGLIDTSLTASVANLLAIAIERHITVFRMQLHTRMSNRRVVVVIVVIWTMAIVMGAIPSVGWNCICDIDHCSNMAPLYSDSYLVFWAIFNLVTFVVMVVLYAHIFGYVRQRTMRMSRHSSGPRRNRDTMMSLLKTVVIVLGAFIVCWTPGLVLLLLDVCCPQCDVLAYEKFFLLLAEFNSAMNPIIYSYRDKEMSATFRQILCCQRNENPNGPTEGSDRSASSLNHTILAGVHSNDHSVV

SEQ ID NO: 113 - DNA, 37 bp, synthetic construct
  source 1..37: mol_type = other DNA
gctagcgctaccggactcagatcccccccccccccdn

SEQ ID NO: 114 - DNA, 23 bp, synthetic construct
  source 1..23: mol_type = other DNA
accytgcatttgaactccttgcc

SEQ ID NO: 115 - DNA, 25 bp, synthetic construct
  source 1..25: mol_type = other DNA
actgccatcaatcttccacttgaca

SEQ ID NO: 116 - DNA, 44 bp, synthetic construct
  source 1..44: mol_type = other DNA
ggtttagtgaaccgtcagatccgctagcgctaccggactcagat

SEQ ID NO: 117 - DNA, 23 bp, synthetic construct
  source 1..23: mol_type = other DNA
ctggacagggatccagagttcca

SEQ ID NO: 118 - DNA, 25 bp, synthetic construct
  source 1..25: mol_type = other DNA
actgaggcacctccagatgttaact

SEQ ID NO: 119 - protein, 351 aa, Homo sapiens
MVIMGQCYYNETIGFFYNNSGKELSSHWRPKDVVVVALGLTVSVLVLLTNLLVIAAIASNRRFHQPIYYLLGNLAAADLFAGVAYLFLMFHTGPRTARLSLEGWFLRQGLLDTSLTASVATLLAIAVERHRSVMAVQLHSRLPRGRVVMLIVGVWVAALGLGLLPAHSWHCLCALDRCSRMAPLLSRSYLAVWALSSLLVFLLMVAVYTRIFFYVRRRVQRMAEHVSCHPRYRETTLSLVKTVVIILGAFVVCWTPGQVVLLLDGLGCESCNVLAVEKYFLLLAEANSLVNAAVYSCRDAEMRRTFRRLLCCACLRQSTRESVHYTSSAQGGASTRIMLPENGHPLMDSTL

SEQ ID NO: 120 - protein, 348 aa, Mus musculus
MGQCYYNETIGFFYNNSGKELSLHWRPKDVVVVALGLTVSVLVLLTNLLVIAAIASNRRFHQPIYYLLGNLAAADLFAGMAYLFLMFHTGPRTARLSIKGWFLRQGLLDTSLTASVATLLAIAVERHRSVMAVQLHSRLPRGRVVTLIVGVWAAALGLGLLPAHFWHCLCDLDSCSRMVPLFSRSYLAAWALSSLLVFLLMVAVYTRIFFYVRRRVERMAEHVSCHPRYRETTLSLVKTVVIILGAFVVCWTPGQVVLLLDGLDCKSCNVLAVEKYFLLLAEANSLVNAVVYSCRDAEMRRTFRRLLCCMCLRWSSHKSARYSASAQTGASTRIMLPENGRPLMDSTL

SEQ ID NO: 121 - protein, 353 aa, Homo sapiens
MNECHYDKHMDFFYNRSNTDTVDDWTGTKLVIVLCVGTFFCLFIFFSNSLVIAAVIKNRKFHFPFYYLLANLAAADFFAGIAYVFLMFNTGPVSKTLTVNRWFLRQGLLDSSLTASLTNLLVIAVERHMSIMRMRVHSNLTKKRVTLLILLVWAIAIFMGAVPTLGWNCLCNISACSSLAPIYSRSYLVFWTVSNLMAFLIMVVVYLRIYVYVKRKTNVLSPHTSGSISRRRTPMKLMKTVMTVLGAFVVCWTPGLVVLLLDGLNCRQCGVQHVKRWFLLLALLNSVVNPIIYSYKDEDMYGTMKKMICCFSQENPERRPSRIPSTVLSRSDTGSQYIEDSISQGAVCNKSTS

SEQ ID NO: 122 - protein, 354 aa, Mus musculus
MNECHYDKRMDFFYNRSNTDTADEWTGTKLVIVLCVGTFFCLFIFFSNSLVIAAVITNRKFHFPFYYLLANLAAADFFAGIAYVFLMFNTGPVSKTLTVNRWFLRQGLLDTSLTASLANLLVIAVERHMSIMRMRVHSNLTKKRVTLLILLVWAIAIFMGAVPTLGWNCLCNISACSSLAPIYSRSYLIFWTVSNLLAFFIMVAVYVRIYMYVKRKTNVLSPHTSGSISRRRAPMKLMKTVMTVLGAFVVCWTPGLVVLLLDGLNCKQCNVQHVKRWFLLLALLNSVMNPIIYSYKDEDMYNTMRKMICCALQDSNTERRPSRNPSTIHSRSETGSQYLEDSISQGPVCNKNGS

SEQ ID NO: 123 - protein, 122 aa, synthetic construct
QVQLVQSGAEVKKPGASVKVSCKASGYTFTSYGISWVRQAPGQGLEWMGEIYPRSGNTYYNEKFKGRVTLTADKSTSTAYMELRSLTSEDTAVYFCARESISRRLGWNFDVWGQGTTVTVSS

SEQ ID NO: 124 - protein, 107 aa, synthetic construct
DIQMTQSPSSLSASVGDTVTITCRASENIYSFLAWYQQKPGKAPKLLIYNAKTLTEGVPSRFSGSGSGTHFSLTINSLQPEDFGIYYCQHHYGPPLTFGQGTKLEIK

SEQ ID NO: 125 - protein, 122 aa, synthetic construct
QVQLQESGPGLVKPSETLSLTCTASGYTFTSYGISWVRQTPGKGLEWIGEIYPRSGNTYYNEKFKGRATLSADKSKNQASLKLKSVTAADTAIYFCARESISRRLGWNFDVWGRGTLVTVSG

SEQ ID NO: 126 - protein, 107 aa, synthetic construct
DIQMTQTPSSLSASVGDRVTITCRASENIYSFLAWYQQKPGEAPKRVVYNAKTLTEGVPSRFSGSGSGTDFTLTISSLQPEDFATYYCQHHYGPPLTFGQGTKLEIK

SEQ ID NO: 127 - protein, 122 aa, synthetic construct
QVQLVQSGAEVKKPGASVKVSCKASGYTFTSYGISWVRQAPGQGLEWIGEIYPRSGNTYYNEKFKGRATLTADKSTSTAYMELRSLRSDDTAVYFCARESISRRLGWNFDVWGTGTTVTVSS

SEQ ID NO: 128 - protein, 107 aa, synthetic construct
DIQMTQSPSSLSASVGDRVTITCRASENIYSFLAWYQQKPGKAPKLVVYNAKTLTEGVPSRFSGSGSGTDFTLTISSLQPEDFATYYCQHHYGPPLTFGAGTKLELK

SEQ ID NO: 129 - protein, 330 aa, Homo sapiens
ASTKGPSVFPLAPSSKSTSGGTAALGCLVKDYFPEPVTVSWNSGALTSGVHTFPAVLQSSGLYSLSSVVTVPSSSLGTQTYICNVNHKPSNTKVDKKVEPKSCDKTHTCPPCPAPEAAGGPSVFLFPPKPKDTLMISRTPEVTCVVVDVSHEDPEVKFNWYVDGVEVHNAKTKPREEQYNSTYRVVSVLTVLHQDWLNGKEYKCKVSNKALPAPIEKTISKAKGQPREPQVYTLPPSRDELTKNQVSLTCLVKGFYPSDIAVEWESNGQPENNYKTTPPVLDSDGSFFLYSKLTVDKSRWQQGNVFSCSVMHEALHNHYTQKSLSLSPGK

SEQ ID NO: 130 - protein, 107 aa, Homo sapiens [sequence omitted]